European Patent Application EP 4 155 402 A1, published March 29, 2023. Title: Modulation of microRNA-335 for the treatment of sodium channelopathies. Applicant: Royal College of Surgeons in Ireland. The sequence listing filed with the application follows.

SEQUENCE LISTING (18 sequences)

SEQ ID NO: 1 - RNA, 23 nt, Homo sapiens
ucaagagcaauaacgaaaaaugu

SEQ ID NO: 2 - RNA, 94 nt, Homo sapiens
uguuuugagcgggggucaagagcaauaacgaaaaauguuugucauaaaccguuuuucauuauugcuccugaccuccucucauuugcuauauuca

SEQ ID NO: 3 - RNA, 98 nt, Mus musculus
ucuuuugggcgggggucaagagcaauaacgaaaaauguuuguuuuucguaaaccguuuuucauuauugcuccugacccccucucauggguuauagcca

SEQ ID NO: 4 - DNA, 21 bp, Artificial Sequence
  ANT-335
catttttcgttattgctcttg

SEQ ID NO: 5 - DNA, 19 bp, Artificial Sequence
  SCR control sequence
taacacgtctatacgccca

SEQ ID NO: 6 - DNA, 42 bp, Artificial Sequence
  U6B primer
cgcaaggatgacacgcaaattcgtgaagcgttccatattttt

SEQ ID NO: 7 - DNA, 20 bp, Artificial Sequence
  B ACTIN FORWARD PRIMER
agcagcagacctgacatcct

SEQ ID NO: 8 - DNA, 20 bp, Artificial Sequence
  B ACTIN REVERSE PRIMER
gtgatgccctttccagacat

SEQ ID NO: 9 - DNA, 20 bp, Artificial Sequence
  SCN1A FORWARD PRIMER
agtttgtggacctgggcaat

SEQ ID NO: 10 - DNA, 20 bp, Artificial Sequence
  SCN1A REVERSE PRIMER
atgaagagctgcaacccgat

SEQ ID NO: 11 - DNA, 20 bp, Artificial Sequence
  SCN2A FORWARD PRIMER
aggaagatgctgtgcggaaa

SEQ ID NO: 12 - DNA, 20 bp, Artificial Sequence
  SCN2A REVERSE PRIMER
acccgacctttgaagctgaa

SEQ ID NO: 13 - DNA, 20 bp, Artificial Sequence
  SCN3A FORWARD PRIMER
tcgcagatgacagccacttt

SEQ ID NO: 14 - DNA, 20 bp, Artificial Sequence
  SCN3A REVERSE PRIMER
ttcccagctgcacgtaatgt

SEQ ID NO: 15 - DNA, 20 bp, Artificial Sequence
  SCN3B FORWARD PRIMER
gttcagcaatgccagcaaca

SEQ ID NO: 16 - DNA, 20 bp, Artificial Sequence
  SCN3B REVERSE PRIMER
atttggagcacaggggacaa

SEQ ID NO: 17 - DNA, 20 bp, Artificial Sequence
  PCDH19 FORWARD PRIMER
attcgcacttcccatccaca

SEQ ID NO: 18 - DNA, 20 bp, Artificial Sequence
  PCDH19 REVERSE PRIMER
agttcagccgcatgttgttg